European Patent Specification EP 3 132 029 B1, published January 28, 2026. Title: MODIFIED TRANSPOSASES FOR IMPROVED INSERTION SEQUENCE BIAS. Applicant: Illumina, Inc. The sequence listing filed with the application follows.

SEQUENCE LISTING (26 sequences)

SEQ ID NO: 1 - protein, 476 aa, Unknown
  Transposase Tn5
MITSALHRAADWAKSVFSSAALGDPRRTARLVNVAAQLAKYSGKSITISSEGSEAMQEGAYRFIRNPNVSAEAIRKAGAMQTVKLAQEFPELLAIEDTTSLSYRHQVAEELGKLGSIQDKSRGWWVHSVLLLEATTFRTVGLLHQEWWMRPDDPADADEKESGKWLAAAATSRLRMGSMMSNVIAVCDREADIHAYLQDKLAHNERFVVRSKHPRKDVESGLYLYDHLKNQPELGGYQISIPQKGVVDKRGKRKNRPARKASLSLRSGRITLKQGNITLNAVLAEEINPPKGETPLKWLLLTSEPVESLAQALRVIDIYTHRWRIEEFHKAWKTGAGAERQRMEEPDNLERMVSILSFVAVRLLQLRESFTLPQALRAQGLLKEAEHVESQSAETVLTPDECQLLGYLDKGKRKRKEKAGSLQWAYMAIARLGGFMDSKRTGIASWGALWEGWEALQSKLDGFLAAKDLMAQGIKI

SEQ ID NO: 2 - protein, 476 aa, Unknown
  Transposase Tn5
  Variant (248)..(248): X = Y, T, K, S, L, A, W, P, G, R, F, H
MITSALHRAADWAKSVFSSAALGDPRRTARLVNVAAQLAKYSGKSITISSEGSEAMQEGAYRFIRNPNVSAEAIRKAGAMQTVKLAQEFPELLAIEDTTSLSYRHQVAEELGKLGSIQDKSRGWWVHSVLLLEATTFRTVGLLHQEWWMRPDDPADADEKESGKWLAAAATSRLRMGSMMSNVIAVCDREADIHAYLQDKLAHNERFVVRSKHPRKDVESGLYLYDHLKNQPELGGYQISIPQKGVVXKRGKRKNRPARKASLSLRSGRITLKQGNITLNAVLAEEINPPKGETPLKWLLLTSEPVESLAQALRVIDIYTHRWRIEEFHKAWKTGAGAERQRMEEPDNLERMVSILSFVAVRLLQLRESFTLPQALRAQGLLKEAEHVESQSAETVLTPDECQLLGYLDKGKRKRKEKAGSLQWAYMAIARLGGFMDSKRTGIASWGALWEGWEALQSKLDGFLAAKDLMAQGIKI

SEQ ID NO: 3 - protein, 476 aa, Unknown
  Transposase Tn5
  Variant (119)..(119): X = L, M, S, A, V
MITSALHRAADWAKSVFSSAALGDPRRTARLVNVAAQLAKYSGKSITISSEGSEAMQEGAYRFIRNPNVSAEAIRKAGAMQTVKLAQEFPELLAIEDTTSLSYRHQVAEELGKLGSIQXKSRGWWVHSVLLLEATTFRTVGLLHQEWWMRPDDPADADEKESGKWLAAAATSRLRMGSMMSNVIAVCDREADIHAYLQDKLAHNERFVVRSKHPRKDVESGLYLYDHLKNQPELGGYQISIPQKGVVDKRGKRKNRPARKASLSLRSGRITLKQGNITLNAVLAEEINPPKGETPLKWLLLTSEPVESLAQALRVIDIYTHRWRIEEFHKAWKTGAGAERQRMEEPDNLERMVSILSFVAVRLLQLRESFTLPQALRAQGLLKEAEHVESQSAETVLTPDECQLLGYLDKGKRKRKEKAGSLQWAYMAIARLGGFMDSKRTGIASWGALWEGWEALQSKLDGFLAAKDLMAQGIKI

SEQ ID NO: 4 - protein, 476 aa, Unknown
  Transposase Tn5
MITSALHRAADWAKSVFSSAALGDPRRTARLVNVAAQLAKYSGKSITISSEGSEAMQEGAYRFIRNPNVSAEAIRKAGAMQTVKLAQEFPELLAIEDTTSLSYRHQVAEELGKLGSIQDKSRGWMVHSVLLLEATTFRTVGLLHQEWWMRPDDPADADEKESGKWLAAAATSRLRMGSMMSNVIAVCDREADIHAYLQDKLAHNERFVVRSKHPRKDVESGLYLYDHLKNQPELGGYQISIPQKGVVDKRGKRKNRPARKASLSLRSGRITLKQGNITLNAVLAEEINPPKGETPLKWLLLTSEPVESLAQALRVIDIYTHRWRIEEFHKAWKTGAGAERQRMEEPDNLERMVSILSFVAVRLLQLRESFTLPQALRAQGLLKEAEHVESQSAETVLTPDECQLLGYLDKGKRKRKEKAGSLQWAYMAIARLGGFMDSKRTGIASWGALWEGWEALQSKLDGFLAAKDLMAQGIKI

SEQ ID NO: 5 - protein, 477 aa, Unknown
  Transposase Tn5
MITSALHRAADWAKSVFSSAALGDPRRTARLVNVAAQLAKYSGKSITISSEGSEAMQEGAYRFIRNPNVSAEAIRKAGAMQTVKLAQEFPELLAIEDTTSLSYRHQVAEELGKLGSIQDKSRGWWVHSVLLLEATTFRTVGLLHQEWWMRPDDPADADEKESGKWLAAAATSRLRMGSMMSNVIAVCDREADIHAYLQDKLAHNERFVVRSKHPRKDVESGLYLYDHLKNQPELGGYQISIPQKGVVDVKRGKRKNRPARKASLSLRSGRITLKQGNITLNAVLAEEINPPKGETPLKWLLLTSEPVESLAQALRVIDIYTHRWRIEEFHKAWKTGAGAERQRMEEPDNLERMVSILSFVAVRLLQLRESFTLPQALRAQGLLKEAEHVESQSAETVLTPDECQLLGYLDKGKRKRKEKAGSLQWAYMAIARLGGFMDSKRTGIASWGALWEGWEALQSKLDGFLAAKDLMAQGIKI

SEQ ID NO: 6 - protein, 476 aa, Unknown
  Transposase Tn5
  Variant (120)..(120): X = Y, F, W, E
MITSALHRAADWAKSVFSSAALGDPRRTARLVNVAAQLAKYSGKSITISSEGSEAMQEGAYRFIRNPNVSAEAIRKAGAMQTVKLAQEFPELLAIEDTTSLSYRHQVAEELGKLGSIQDXSRGWWVHSVLLLEATTFRTVGLLHQEWWMRPDDPADADEKESGKWLAAAATSRLRMGSMMSNVIAVCDREADIHAYLQDKLAHNERFVVRSKHPRKDVESGLYLYDHLKNQPELGGYQISIPQKGVVDKRGKRKNRPARKASLSLRSGRITLKQGNITLNAVLAEEINPPKGETPLKWLLLTSEPVESLAQALRVIDIYTHRWRIEEFHKAWKTGAGAERQRMEEPDNLERMVSILSFVAVRLLQLRESFTLPQALRAQGLLKEAEHVESQSAETVLTPDECQLLGYLDKGKRKRKEKAGSLQWAYMAIARLGGFMDSKRTGIASWGALWEGWEALQSKLDGFLAAKDLMAQGIKI

SEQ ID NO: 7 - protein, 476 aa, Unknown
  Transposase Tn5
  Variant (119)..(119): X = L, M, S, A, V
  Variant (120)..(120): X = Y, F, W, E
  Variant (248)..(248): X = Y, T, K, S, L, A, W, P, G, R, F, H
MITSALHRAADWAKSVFSSAALGDPRRTARLVNVAAQLAKYSGKSITISSEGSEAMQEGAYRFIRNPNVSAEAIRKAGAMQTVKLAQEFPELLAIEDTTSLSYRHQVAEELGKLGSIQXXSRGWMVHSVLLLEATTFRTVGLLHQEWWMRPDDPADADEKESGKWLAAAATSRLRMGSMMSNVIAVCDREADIHAYLQDKLAHNERFVVRSKHPRKDVESGLYLYDHLKNQPELGGYQISIPQKGVVXKRGKRKNRPARKASLSLRSGRITLKQGNITLNAVLAEEINPPKGETPLKWLLLTSEPVESLAQALRVIDIYTHRWRIEEFHKAWKTGAGAERQRMEEPDNLERMVSILSFVAVRLLQLRESFTLPQALRAQGLLKEAEHVESQSAETVLTPDECQLLGYLDKGKRKRKEKAGSLQWAYMAIARLGGFMDSKRTGIASWGALWEGWEALQSKLDGFLAAKDLMAQGIKI

SEQ ID NO: 8 - protein, 476 aa, Unknown
  Transposase Tn5
MITSALHRAADWAKSVFSSAALGDPRRTARLVNVAAQLAKYSGKSITISSEGSEAMQEGAYRFIRNPNVSAEAIRKAGAMQTVKLAQEFPELLAIEDTTSLSYRHQVAEELGKLGSIQDKSRGWWVHSVLLLEATTFRTVGLLHQEWWMRPDDPADADEKESGKWLAAAATSRLRMGSMMSNVIAVCDREADIHAYLQDKLAHNERFVVRSRHRRKDVESGLYLYDHLKNQPELGGYQISIPQKGVVDKRGKRKNRPARKASLSLRSGRITLKQGNITLNAVLAEEINPPKGETPLKWLLLTSEPVESLAQALRVIDIYTHRWRIEEFHKAWKTGAGVERQRMEEPDNLERMVSILSFVAVRLLQLRESFTLPQALRAQGLLKEAEHVESQSAETVLTPDECQLLGYLDKGKRKRKEKAGSLQWAYMAIARLGGFMDSKRTGIASWGALWEGWEALQSKLDGFLAAKDLMAQGIKI

SEQ ID NO: 9 - protein, 476 aa, Unknown
  Transposase Tn5
MITSALHRAADWAKSVFSSAALGDPRRTARLVNVAAQLAKYSGKSITISSEGSEAMQEGAYRFIRNPNVSAEAIRKAGAMQTVKLAQEFPELLAIEDTTSLSYRHQVAEELGKLGSIQDKSRGWWVHSVLLLEATTFRTVGLLHQEWWMRPDDPADADEKESGKWLAAAATSRLRMGSMMSNVIAVCDREADIHAYLQDKLAHNERFVVRSRHRRKDVESGLYLYDHLKNQPELGGYQISIPQKGVVDKRRKRKNRPARKASLSLRSGRITLKQGNITLNAVLAEEINPPKGETPLKWLLLTSEPVESLAQALRVIDIYTHRWRIEEFHKAWKTGAGVERQRMEEPDNLERMVSILSFVAVRLLQLRESFTLPQALRAQGLLKEAEHVESQSAETVLTPDECQLLGYLDKGKRKRKEKAGSLQWAYMAIARLGGFMDSKRTGIASWGALWEGWEALQSKLDGFLAAKDLMAQGIKI

SEQ ID NO: 10 - protein, 476 aa, Unknown
  Transposase Tn5
MITSALHRAADWAKSVFSSAALGDPRRTARLVNVAAQLAKYSGKSITISSEGSEAMQEGAYRFIRNPNVSAEAIRKAGAMQTVKLAQEFPELLAIEDTTSLSYRHQVAEELGKLGSIQDKSRGWWVHSVLLLEATTFRTVGLLHQQWWMRPDDPADADEKESGKWLAAAATSRLRMGSMMSNVIAVCDRGADIHAYLQDKLAHNERFVVRSKHPRKDVESGLYLYDHLKNQPELGGYQISIPQKGVVDKRRKRKNRPARKASLSLRSGRITLKQGNITLNAVLAEEINPPKGETPLKWLLLTSEPVESLAQALRVIDIYTHRWRIEEFHKAWKTGAGAERQRMEEPDNLERMVSILSFVAVRLLQLRESFTLPQALRAQGLLKEAEHVESQSAETVLTPDECQLLGYLDKGKRKRKEKAGSLQWAYMAIARLGGFMDSKRTGIASWGALWEGWEALQSKLDGFLAAKDLMAQGIKI

SEQ ID NO: 11 - protein, 476 aa, Unknown
  Transposase Tn5
MITSALHRAADWAKSVFSSAALGDPRRTARLVNVAAQLAKYSGKSITISSEGSKAAQEGAYRFIRNPNVSAEAIRKAGAMQTVKLAQEFPELLAIEDTTSLSYRHQVAEELGKLGSIQDKSRGWWVHSVLLLEATTFRTVGLLHQEWWMRPDDPADADEKESGKWLAAAATSRLRMGSMMSNVIAVCDREADIHAYLQDKLAHNERFVVRSKHPRKDVESGLYLYDHLKNQPELGGYQISIPQKGVVDKRGKRKNRPARKASLSLRSGRITLKQGNITLNAVLAEEINPPKGETPLKWLLLTSEPVESLAQALRVIDIYTHRWRIEEFHKAWKTGAGAERQRMEEPDNLERMVSILSFVAVRLLQLRESFTPPQALRAQGLLKEAEHVESQSAETVLTPDECQLLGYLDKGKRKRKEKAGSLQWAYMAIARLGGFMDSKRTGIASWGALWEGWEALQSKLDGFLAAKDLMAQGIKI

SEQ ID NO: 12 - protein, 476 aa, Unknown
  Transposase Tn5
  VARIANT (248)..(248): X = Y, T, K, S, L, A, W, P, G, R, F, H
MITSALHRAADWAKSVFSSAALGDPRRTARLVNVAAQLAKYSGKSITISSEGSKAAQEGAYRFIRNPNVSAEAIRKAGAMQTVKLAQEFPELLAIEDTTSLSYRHQVAEELGKLGSIQDKSRGWWVHSVLLLEATTFRTVGLLHQEWWMRPDDPADADEKESGKWLAAAATSRLRMGSMMSNVIAVCDREADIHAYLQDKLAHNERFVVRSKHPRKDVESGLYLYDHLKNQPELGGYQISIPQKGVVXKRGKRKNRPARKASLSLRSGRITLKQGNITLNAVLAEEINPPKGETPLKWLLLTSEPVESLAQALRVIDIYTHRWRIEEFHKAWKTGAGAERQRMEEPDNLERMVSILSFVAVRLLQLRESFTPPQALRAQGLLKEAEHVESQSAETVLTPDECQLLGYLDKGKRKRKEKAGSLQWAYMAIARLGGFMDSKRTGIASWGALWEGWEALQSKLDGFLAAKDLMAQGIKI

SEQ ID NO: 13 - protein, 476 aa, Unknown
  Transposase Tn5
  Variant (119)..(119): X = L, M, S, A, V
MITSALHRAADWAKSVFSSAALGDPRRTARLVNVAAQLAKYSGKSITISSEGSKAAQEGAYRFIRNPNVSAEAIRKAGAMQTVKLAQEFPELLAIEDTTSLSYRHQVAEELGKLGSIQXKSRGWWVHSVLLLEATTFRTVGLLHQEWWMRPDDPADADEKESGKWLAAAATSRLRMGSMMSNVIAVCDREADIHAYLQDKLAHNERFVVRSKHPRKDVESGLYLYDHLKNQPELGGYQISIPQKGVVDKRGKRKNRPARKASLSLRSGRITLKQGNITLNAVLAEEINPPKGETPLKWLLLTSEPVESLAQALRVIDIYTHRWRIEEFHKAWKTGAGAERQRMEEPDNLERMVSILSFVAVRLLQLRESFTPPQALRAQGLLKEAEHVESQSAETVLTPDECQLLGYLDKGKRKRKEKAGSLQWAYMAIARLGGFMDSKRTGIASWGALWEGWEALQSKLDGFLAAKDLMAQGIKI

SEQ ID NO: 14 - protein, 476 aa, Unknown
  Transposase Tn5
MITSALHRAADWAKSVFSSAALGDPRRTARLVNVAAQLAKYSGKSITISSEGSKAAQEGAYRFIRNPNVSAEAIRKAGAMQTVKLAQEFPELLAIEDTTSLSYRHQVAEELGKLGSIQDKSRGWMVHSVLLLEATTFRTVGLLHQEWWMRPDDPADADEKESGKWLAAAATSRLRMGSMMSNVIAVCDREADIHAYLQDKLAHNERFVVRSKHPRKDVESGLYLYDHLKNQPELGGYQISIPQKGVVDKRGKRKNRPARKASLSLRSGRITLKQGNITLNAVLAEEINPPKGETPLKWLLLTSEPVESLAQALRVIDIYTHRWRIEEFHKAWKTGAGAERQRMEEPDNLERMVSILSFVAVRLLQLRESFTPPQALRAQGLLKEAEHVESQSAETVLTPDECQLLGYLDKGKRKRKEKAGSLQWAYMAIARLGGFMDSKRTGIASWGALWEGWEALQSKLDGFLAAKDLMAQGIKI

SEQ ID NO: 15 - protein, 477 aa, Unknown
  Transposase Tn5
MITSALHRAADWAKSVFSSAALGDPRRTARLVNVAAQLAKYSGKSITISSEGSKAAQEGAYRFIRNPNVSAEAIRKAGAMQTVKLAQEFPELLAIEDTTSLSYRHQVAEELGKLGSIQDKSRGWWVHSVLLLEATTFRTVGLLHQEWWMRPDDPADADEKESGKWLAAAATSRLRMGSMMSNVIAVCDREADIHAYLQDKLAHNERFVVRSKHPRKDVESGLYLYDHLKNQPELGGYQISIPQKGVVDVKRGKRKNRPARKASLSLRSGRITLKQGNITLNAVLAEEINPPKGETPLKWLLLTSEPVESLAQALRVIDIYTHRWRIEEFHKAWKTGAGAERQRMEEPDNLERMVSILSFVAVRLLQLRESFTPPQALRAQGLLKEAEHVESQSAETVLTPDECQLLGYLDKGKRKRKEKAGSLQWAYMAIARLGGFMDSKRTGIASWGALWEGWEALQSKLDGFLAAKDLMAQGIKI

SEQ ID NO: 16 - protein, 476 aa, Unknown
  Transposase Tn5
  Variant (120)..(120): X = Y, F, W, E
MITSALHRAADWAKSVFSSAALGDPRRTARLVNVAAQLAKYSGKSITISSEGSKAAQEGAYRFIRNPNVSAEAIRKAGAMQTVKLAQEFPELLAIEDTTSLSYRHQVAEELGKLGSIQDXSRGWWVHSVLLLEATTFRTVGLLHQEWWMRPDDPADADEKESGKWLAAAATSRLRMGSMMSNVIAVCDREADIHAYLQDKLAHNERFVVRSKHPRKDVESGLYLYDHLKNQPELGGYQISIPQKGVVDKRGKRKNRPARKASLSLRSGRITLKQGNITLNAVLAEEINPPKGETPLKWLLLTSEPVESLAQALRVIDIYTHRWRIEEFHKAWKTGAGAERQRMEEPDNLERMVSILSFVAVRLLQLRESFTPPQALRAQGLLKEAEHVESQSAETVLTPDECQLLGYLDKGKRKRKEKAGSLQWAYMAIARLGGFMDSKRTGIASWGALWEGWEALQSKLDGFLAAKDLMAQGIKI

SEQ ID NO: 17 - protein, 476 aa, Unknown
  Transposase Tn5
  Variant (119)..(119): X = L, M, S, A, V
  Variant (120)..(120): X = Y, F, W, E
  Variant (248)..(248): X = Y, T, K, S, L, A, W, P, G, R, F, H
MITSALHRAADWAKSVFSSAALGDPRRTARLVNVAAQLAKYSGKSITISSEGSKAAQEGAYRFIRNPNVSAEAIRKAGAMQTVKLAQEFPELLAIEDTTSLSYRHQVAEELGKLGSIQXXSRGWMVHSVLLLEATTFRTVGLLHQEWWMRPDDPADADEKESGKWLAAAATSRLRMGSMMSNVIAVCDREADIHAYLQDKLAHNERFVVRSKHPRKDVESGLYLYDHLKNQPELGGYQISIPQKGVVXKRGKRKNRPARKASLSLRSGRITLKQGNITLNAVLAEEINPPKGETPLKWLLLTSEPVESLAQALRVIDIYTHRWRIEEFHKAWKTGAGAERQRMEEPDNLERMVSILSFVAVRLLQLRESFTPPQALRAQGLLKEAEHVESQSAETVLTPDECQLLGYLDKGKRKRKEKAGSLQWAYMAIARLGGFMDSKRTGIASWGALWEGWEALQSKLDGFLAAKDLMAQGIKI

SEQ ID NO: 18 - protein, 476 aa, Unknown
  Transposase Tn5
MITSALHRAADWAKSVFSSAALGDPRRTARLVNVAAQLAKYSGKSITISSEGSKAAQEGAYRFIRNPNVSAEAIRKAGAMQTVKLAQEFPELLAIEDTTSLSYRHQVAEELGKLGSIQDKSRGWWVHSVLLLEATTFRTVGLLHQEWWMRPDDPADADEKESGKWLAAAATSRLRMGSMMSNVIAVCDREADIHAYLQDKLAHNERFVVRSRHRRKDVESGLYLYDHLKNQPELGGYQISIPQKGVVDKRGKRKNRPARKASLSLRSGRITLKQGNITLNAVLAEEINPPKGETPLKWLLLTSEPVESLAQALRVIDIYTHRWRIEEFHKAWKTGAGVERQRMEEPDNLERMVSILSFVAVRLLQLRESFTPPQALRAQGLLKEAEHVESQSAETVLTPDECQLLGYLDKGKRKRKEKAGSLQWAYMAIARLGGFMDSKRTGIASWGALWEGWEALQSKLDGFLAAKDLMAQGIKI

SEQ ID NO: 19 - protein, 476 aa, Unknown
  Transposase Tn5
MITSALHRAADWAKSVFSSAALGDPRRTARLVNVAAQLAKYSGKSITISSEGSKAAQEGAYRFIRNPNVSAEAIRKAGAMQTVKLAQEFPELLAIEDTTSLSYRHQVAEELGKLGSIQDKSRGWWVHSVLLLEATTFRTVGLLHQEWWMRPDDPADADEKESGKWLAAAATSRLRMGSMMSNVIAVCDREADIHAYLQDKLAHNERFVVRSRHRRKDVESGLYLYDHLKNQPELGGYQISIPQKGVVDKRRKRKNRPARKASLSLRSGRITLKQGNITLNAVLAEEINPPKGETPLKWLLLTSEPVESLAQALRVIDIYTHRWRIEEFHKAWKTGAGVERQRMEEPDNLERMVSILSFVAVRLLQLRESFTPPQALRAQGLLKEAEHVESQSAETVLTPDECQLLGYLDKGKRKRKEKAGSLQWAYMAIARLGGFMDSKRTGIASWGALWEGWEALQSKLDGFLAAKDLMAQGIKI

SEQ ID NO: 20 - protein, 476 aa, Unknown
  Transposase Tn5
MITSALHRAADWAKSVFSSAALGDPRRTARLVNVAAQLAKYSGKSITISSEGSKAAQEGAYRFIRNPNVSAEAIRKAGAMQTVKLAQEFPELLAIEDTTSLSYRHQVAEELGKLGSIQDKSRGWWVHSVLLLEATTFRTVGLLHQQWWMRPDDPADADEKESGKWLAAAATSRLRMGSMMSNVIAVCDRGADIHAYLQDKLAHNERFVVRSKHPRKDVESGLYLYDHLKNQPELGGYQISIPQKGVVDKRRKRKNRPARKASLSLRSGRITLKQGNITLNAVLAEEINPPKGETPLKWLLLTSEPVESLAQALRVIDIYTHRWRIEEFHKAWKTGAGAERQRMEEPDNLERMVSILSFVAVRLLQLRESFTPPQALRAQGLLKEAEHVESQSAETVLTPDECQLLGYLDKGKRKRKEKAGSLQWAYMAIARLGGFMDSKRTGIASWGALWEGWEALQSKLDGFLAAKDLMAQGIKI

SEQ ID NO: 21 - protein, 10 aa, Unknown
  Transposase Tn5
  Variant (1)..(1): x= W, R, K, P, T
  Variant (2)..(2): x= W, N, V, K, M
  Variant (3)..(3): x= V, F, I, T, L
  Variant (4)..(4): x= H, L, W, C
  Variant (5)..(5): x= S, G, V, F
  Variant (6)..(6): x= V, A, W
  Variant (7)..(7): x= L, T, V, Q, W
  Variant (8)..(8): x= L, H, D
  Variant (9)..(9): x= L, H, V
  Variant (10)..(10): x= E, Y, A, K, Q
XXXXXXXXXX

SEQ ID NO: 22 - DNA, 852 bp, Escherichia coli
atggctgaaattaccgcatccctggtaaaagagctgcgtgagcgtactggcgcaggcatgatggattgcaaaaaagcactgactgaagctaacggcgacatcgagctggcaatcgaaaacatgcgtaagtccggtgctattaaagcagcgaaaaaagcaggcaacgttgctgctgacggcgtgatcaaaaccaaaatcgacggcaactacggcatcattctggaagttaactgccagactgacttcgttgcaaaagacgctggtttccaggcgttcgcagacaaagttctggacgcagctgttgctggcaaaatcactgacgttgaagttctgaaagcacagttcgaagaagaacgtgttgcgctggtagcgaaaattggtgaaaacatcaacattcgccgcgttgctgcgctggaaggcgacgttctgggttcttatcagcacggtgcgcgtatcggcgttctggttgctgctaaaggcgctgacgaagagctggttaaacacatcgctatgcacgttgctgcaagcaagccagaattcatcaaaccggaagacgtatccgctgaagtggtagaaaaagaataccaggtacagctggatatcgcgatgcagtctggtaagccgaaagaaatcgcagagaaaatggttgaaggccgcatgaagaaattcaccggcgaagtttctctgaccggtcagccgttcgttatggaaccaagcaaaactgttggtcagctgctgaaagagcataacgctgaagtgactggcttcatccgcttcgaagtgggtgaaggcatcgagaaagttgagactgactttgcagcagaagttgctgcgatgtccaagcagtcttaa

SEQ ID NO: 23 - protein, 283 aa, Escherichia coli
MAEITASLVKELRERTGAGMMDCKKALTEANGDIELAIENMRKSGAIKAAKKAGNVAADGVIKTKIDGNYGIILEVNCQTDFVAKDAGFQAFADKVLDAAVAGKITDVEVLKAQFEEERVALVAKIGENINIRRVAALEGDVLGSYQHGARIGVLVAAKGADEELVKHIAMHVAASKPEFIKPEDVSAEVVEKEYQVQLDIAMQSGKPKEIAEKMVEGRMKKFTGEVSLTGQPFVMEPSKTVGQLLKEHNAEVTGFIRFEVGEGIEKVETDFAAEVAAMSKQS

SEQ ID NO: 24 - DNA, 2283 bp, Unknown
  TS-Tn5 nucleic acid sequence
atggctgaaattaccgcatccctggtaaaagagctgcgtgagcgtactggcgcaggcatgatggattgcaaaaaagcactgactgaagctaacggcgacatcgagctggcaatcgaaaacatgcgtaagtccggtgctattaaagcagcgaaaaaagcaggcaacgttgctgctgacggcgtgatcaaaaccaaaatcgacggcaactacggcatcattctggaagttaactgccagactgacttcgttgcaaaagacgctggtttccaggcgttcgcagacaaagttctggacgcagctgttgctggcaaaatcactgacgttgaagttctgaaagcacagttcgaagaagaacgtgttgcgctggtagcgaaaattggtgaaaacatcaacattcgccgcgttgctgcgctggaaggcgacgttctgggttcttatcagcacggtgcgcgtatcggcgttctggttgctgctaaaggcgctgacgaagagctggttaaacacatcgctatgcacgttgctgcaagcaagccagaattcatcaaaccggaagacgtatccgctgaagtggtagaaaaagaataccaggtacagctggatatcgcgatgcagtctggtaagccgaaagaaatcgcagagaaaatggttgaaggccgcatgaagaaattcaccggcgaagtttctctgaccggtcagccgttcgttatggaaccaagcaaaactgttggtcagctgctgaaagagcataacgctgaagtgactggcttcatccgcttcgaagtgggtgaaggcatcgagaaagttgagactgactttgcagcagaagttgctgcgatgtccaagcagtctggtaccataacttctgctcttcatcgtgcggccgactgggctaaatctgtgttctcttcggcggcgctgggtgatcctcgccgtactgcccgcttggttaacgtcgccgcccaattggcaaaatattctggtaaatcaataaccatctcatcagagggtagtaaagccgcccaggaaggcgcttaccgatttatccgcaatcccaacgtttctgccgaggcgatcagaaaggctggcgccatgcaaacagtcaagttggctcaggagtttcccgaactgctggccattgaggacaccacctctttgagttatcgccaccaggtcgccgaagagcttggcaagctgggctctattcaggataaatcccgcggatggtgggttcactccgttctcttgctcgaggccaccacattccgcaccgtaggattactgcatcaggagtggtggatgcgcccggatgaccctgccgatgcggatgaaaaggagagtggcaaatggctggcagcggccgcaactagccggttacgcatgggcagcatgatgagcaacgtgattgcggtctgtgaccgcgaagccgatattcatgcttatctgcaggacaaactggcgcataacgagcgcttcgtggtgcgctccaagcacccacgcaaggacgtagagtctgggttgtatctgtacgaccatctgaagaaccaaccggagttgggtggctatcagatcagcattccgcaaaagggcgtggtggataaacgcggtaaacgtaaaaatcgaccagcccgcaaggcgagcttgagcctgcgcagtgggcgcatcacgctaaaacaggggaatatcacgctcaacgcggtgctggccgaggagattaacccgcccaagggtgagaccccgttgaaatggttgttgctgaccagcgaaccggtcgagtcgctagcccaagccttgcgcgtcatcgacatttatacccatcgctggcggatcgaggagttccataaggcatggaaaaccggagcaggagccgagaggcaacgcatggaggagccggataatctggagcggatggtctcgatcctctcgtttgttgcggtcaggctgttacagctcagagaaagcttcacgccgccgcaagcactcagggcgcaagggctgctaaaggaagcggaacacgtagaaagccagtccgcagaaacggtgctgaccccggatgaatgtcagctactgggctatctggacaagggaaaacgcaagcgcaaagagaaagcaggtagcttgcagtgggcttacatggcgatagctagactgggcggttttatggacagcaagcgaaccggaattgccagctggggcgccctctgggaaggttgggaagccctgcaaagtaaactggatggctttcttgccgccaaggatctgatggcgcaggggatcaagatctga

SEQ ID NO: 25 - protein, 760 aa, Unknown
  TS-Tn5 Fusion Protein Amino Acid Sequence
MAEITASLVKELRERTGAGMMDCKKALTEANGDIELAIENMRKSGAIKAAKKAGNVAADGVIKTKIDGNYGIILEVNCQTDFVAKDAGFQAFADKVLDAAVAGKITDVEVLKAQFEEERVALVAKIGENINIRRVAALEGDVLGSYQHGARIGVLVAAKGADEELVKHIAMHVAASKPEFIKPEDVSAEVVEKEYQVQLDIAMQSGKPKEIAEKMVEGRMKKFTGEVSLTGQPFVMEPSKTVGQLLKEHNAEVTGFIRFEVGEGIEKVETDFAAEVAAMSKQSGTITSALHRAADWAKSVFSSAALGDPRRTARLVNVAAQLAKYSGKSITISSEGSKAAQEGAYRFIRNPNVSAEAIRKAGAMQTVKLAQEFPELLAIEDTTSLSYRHQVAEELGKLGSIQDKSRGWWVHSVLLLEATTFRTVGLLHQEWWMRPDDPADADEKESGKWLAAAATSRLRMGSMMSNVIAVCDREADIHAYLQDKLAHNERFVVRSKHPRKDVESGLYLYDHLKNQPELGGYQISIPQKGVVDKRGKRKNRPARKASLSLRSGRITLKQGNITLNAVLAEEINPPKGETPLKWLLLTSEPVESLAQALRVIDIYTHRWRIEEFHKAWKTGAGAERQRMEEPDNLERMVSILSFVAVRLLQLRESFTPPQALRAQGLLKEAEHVESQSAETVLTPDECQLLGYLDKGKRKRKEKAGSLQWAYMAIARLGGFMDSKRTGIASWGALWEGWEALQSKLDGFLAAKDLMAQGIKI

SEQ ID NO: 26 - protein, 760 aa, unknown
  TS-Tn mutant protein
MAEITASLVKELRERTGAGMMDCKKALTEANGDIELAIENMRKSGAIKAAKKAGNVAADGVIKTKIDGNYGIILEVNCQTDFVAKDAGFQAFADKVLDAAVAGKITDVEVLKAQFEEERVALVAKIGENINIRRVAALEGDVLGSYQHGARIGVLVAAKGADEELVKHIAMHVAASKPEFIKPEDVSAEVVEKEYQVQLDIAMQSGKPKEIAEKMVEGRMKKFTGEVSLTGQPFVMEPSKTVGQLLKEHNAEVTGFIRFEVGEGIEKVETDFAAEVAAMSKQSGTITSALHRAADWAKSVFSSAALGDPRRTARLVNVAAQLAKYSGKSITISSEGSKAAQEGAYRFIRNPNVSAEAIRKAGAMQTVKLAQEFPELLAIEDTTSLSYRHQVAEELGKLGSIQDKSRGWWVHSVLLLEATTFRTVGLLHQEWWMRPDDPADADEKESGKWLAAAATSRLRMGSMMSNVIAVCDREADIHAYLQDKLAHNERFVVRSRHRRKDVESGLYLYDHLKNQPELGGYQISIPQKGVVDKRRKRKNRPARKASLSLRSGRITLKQGNITLNAVLAEEINPPKGETPLKWLLLTSEPVESLAQALRVIDIYTHRWRIEEFHKAWKTGAGVERQRMEEPDNLERMVSILSFVAVRLLQLRESFTPPQALRAQGLLKEAEHVESQSAETVLTPDECQLLGYLDKGKRKRKEKAGSLQWAYMAIARLGGFMDSKRTGIASWGALWEGWEALQSKLDGFLAAKDLMAQGIKI